European Patent Specification EP 3 775 162 B1, published August 6, 2025. Title: MATURE AIRWAY ORGANOIDS, METHODS OF MAKING AND USES THEREOF. Applicant: The University of Hong Kong Koninklijke Nederlandse Akademie Van Wetenschappen. The sequence listing filed with the application follows.

SEQUENCE LISTING (24 sequences)

SEQ ID NO: 1 - DNA, 20 bp, Artificial Sequence
  synthetic sequence
cagactcaatttagtgagcc

SEQ ID NO: 2 - DNA, 18 bp, Artificial Sequence
  synthetic sequence
ctgctggtccatgctgtt

SEQ ID NO: 3 - DNA, 21 bp, Artificial Sequence
  synthetic sequence
gaggaatgcagactcagtgga

SEQ ID NO: 4 - DNA, 21 bp, Artificial Sequence
  synthetic sequence
tagcttccactgctacctccg

SEQ ID NO: 5 - DNA, 20 bp, Artificial Sequence
  synthetic sequence
tcgtatgccacgctcatctg

SEQ ID NO: 6 - DNA, 20 bp, Artificial Sequence
  synthetic sequence
cggattgaattctgccaggt

SEQ ID NO: 7 - DNA, 20 bp, Artificial Sequence
  synthetic sequence
gctgcaaacccaatttagga

SEQ ID NO: 8 - DNA, 22 bp, Artificial Sequence
  synthetic sequence
tgctcatcaagttcagaaagga

SEQ ID NO: 9 - DNA, 20 bp, Artificial Sequence
  synthetic sequence
cctacaaagctgaggcctgt

SEQ ID NO: 10 - DNA, 20 bp, Artificial Sequence
  synthetic sequence
gaccctcctctcaatggtgc

SEQ ID NO: 11 - DNA, 24 bp, Artificial Sequence
  synthetic sequence
agcatcattaagctcatggaaaaa

SEQ ID NO: 12 - DNA, 20 bp, Artificial Sequence
  synthetic sequence
gtggactcaaagcatggcag

SEQ ID NO: 13 - DNA, 20 bp, Artificial Sequence
  synthetic sequence
aactgctggaggcgctatca

SEQ ID NO: 14 - DNA, 20 bp, Artificial Sequence
  synthetic sequence
tgtccttttcacgggtcact

SEQ ID NO: 15 - DNA, 20 bp, Artificial Sequence
  synthetic sequence
ctttgaactcagggtcacca

SEQ ID NO: 16 - DNA, 20 bp, Artificial Sequence
  synthetic sequence
tagtactgagccggatgcac

SEQ ID NO: 17 - DNA, 20 bp, Artificial Sequence
  synthetic sequence
tgcttcaggaaacataccga

SEQ ID NO: 18 - DNA, 20 bp, Artificial Sequence
  synthetic sequence
ctggagtgagctcctcatca

SEQ ID NO: 19 - DNA, 20 bp, Artificial Sequence
  synthetic sequence
tacacaggaatacaggactt

SEQ ID NO: 20 - DNA, 18 bp, Artificial Sequence
  synthetic sequence
ctcacaccactaccatct

SEQ ID NO: 21 - DNA, 20 bp, Artificial Sequence
  synthetic sequence
ctaggatgagcagctgtgga

SEQ ID NO: 22 - DNA, 20 bp, Artificial Sequence
  synthetic sequence
aagaatttgaagcgcacctt

SEQ ID NO: 23 - DNA, 21 bp, Artificial Sequence
  synthetic sequence
cttctaaccgaggtcgaaacg

SEQ ID NO: 24 - DNA, 22 bp, Artificial Sequence
  synthetic sequence
ggcattttggacaaakcgtcta